European Patent Specification EP 3 693 368 B1, published December 6, 2023. Title: Heterocyclic compound. Applicant: TAKEDA PHARMACEUTICAL COMPANY LIMITED. The sequence listing filed with the application follows.

SEQUENCE LISTING (4 sequences)

SEQ ID NO: 1 - DNA, 42 bp, Artificial
  Forward primer for GluR1 flip cDNA
actgaattcgccaccatgcagcacatttttgccttcttctgc

SEQ ID NO: 2 - DNA, 32 bp, Artificial
  Reverse primer for GluR1 flip cDNA
ccgcggccgcttacaatcccgtggctcccaag

SEQ ID NO: 3 - DNA, 41 bp, Artificial
  Forward primer for stargazin cDNA
ggtctcgaggccaccatggggctgtttgatcgaggtgttca

SEQ ID NO: 4 - DNA, 40 bp, Artificial
  Reverse primer for stargazin cDNA
gttggatccttatacgggggtggtccggcggttggctgtg